European Patent Specification EP 3 591 045 B1, published July 17, 2024. Title: COMPOSITIONS FOR LINKING DNA-BINDING DOMAINS AND CLEAVAGE DOMAINS. Applicant: SANGAMO THERAPEUTICS, INC. The sequence listing filed with the application follows.

SEQUENCE LISTING (312 sequences)

SEQ ID NO: 1 - protein, 353 aa, Artificial Sequence
  Description of Artificial Sequence: Synthetic polypeptide
MDYKDHDGDYKDHDIDYKDDDDKMAPKKKRKVGIHGVPAAMAERPFQCRICMRNFSDRSNLSRHIRTHTGEKPFACDICGRKFAISSNLNSHTKIHTGSQKPFQCRICMRNFSRSDNLARHIRTHTGEKPFACDICGRKFATSGNLTRHTKIHLRGSQLVKSELEEKKSELRHKLKYVPHEYIELIEIARNSTQDRILEMKVMEFFMKVYGYRGKHLGGSRKPDGAIYTVGSPIDYGVIVDTKAYSGGYNLPIGQADEMQRYVEENQTRNKHINPNEWWKVYPSSVTEFKFLFVSGHFKGNYKAQLTRLNHITNCNGAVLSVEELLIGGEMIKAGTLTLEEVRRKFNNGEINF

SEQ ID NO: 2 - protein, 14 aa, Artificial Sequence
  Description of Artificial Sequence: Synthetic peptide
  misc_feature (1)..(1): May or may not be present
NGICPPPRPRTSPP

SEQ ID NO: 3 - protein, 14 aa, Artificial Sequence
  Description of Artificial Sequence: Synthetic peptide
  misc_feature (1)..(1): May or may not be present
TGTAPIEIPPEVYP

SEQ ID NO: 4 - protein, 15 aa, Artificial Sequence
  Description of Artificial Sequence: Synthetic peptide
  misc_feature (1)..(1): May or may not be present
NGSYAPMPPLALASP

SEQ ID NO: 5 - protein, 15 aa, Artificial Sequence
  Description of Artificial Sequence: Synthetic peptide
  misc_feature (1)..(1): May or may not be present
PGIYTAPTSRPTVPP

SEQ ID NO: 6 - protein, 16 aa, Artificial Sequence
  Description of Artificial Sequence: Synthetic peptide
  misc_feature (1)..(1): May or may not be present
NGSQTPKRFQPTHPSA

SEQ ID NO: 7 - protein, 12 aa, Artificial Sequence
  Description of Artificial Sequence: Synthetic peptide
  misc_feature (1)..(1): May or may not be present
HLPKPANPFPLD

SEQ ID NO: 8 - protein, 14 aa, Artificial Sequence
  Description of Artificial Sequence: Synthetic peptide
  misc_feature (1)..(1): May or may not be present
HRDGPRNLPPTSPP

SEQ ID NO: 9 - protein, 15 aa, Artificial Sequence
  Description of Artificial Sequence: Synthetic peptide
  misc_feature (1)..(1): May or may not be present
HRLPDSPTALAPDTL

SEQ ID NO: 10 - protein, 16 aa, Artificial Sequence
  Description of Artificial Sequence: Synthetic peptide
  misc_feature (1)..(4): May or may not be present
DPNSPISRARPLNPHP

SEQ ID NO: 11 - protein, 19 aa, Artificial Sequence
  Description of Artificial Sequence: Synthetic peptide
  misc_feature (1)..(1): May or may not be present
YGPRPTPRLRCPIDSLIFR

SEQ ID NO: 12 - protein, 10 aa, Artificial Sequence
  Description of Artificial Sequence: Synthetic peptide
  misc_feature (1)..(1): May or may not be present
HCPASRPIHP

SEQ ID NO: 13 - protein, 11 aa, Artificial Sequence
  Description of Artificial Sequence: Synthetic peptide
  misc_feature (1)..(1): May or may not be present
GLQSLIPQQLL

SEQ ID NO: 14 - protein, 12 aa, Artificial Sequence
  Description of Artificial Sequence: Synthetic peptide
  misc_feature (1)..(1): May or may not be present
GLQPTVNHEYNN

SEQ ID NO: 15 - protein, 13 aa, Artificial Sequence
  Description of Artificial Sequence: Synthetic peptide
  misc_feature (1)..(1): May or may not be present
PANIHSLSSPPPL

SEQ ID NO: 16 - protein, 15 aa, Artificial Sequence
  Description of Artificial Sequence: Synthetic peptide
  misc_feature (1)..(1): May or may not be present
PAGLNTPCSPRSRSN

SEQ ID NO: 17 - protein, 8 aa, Artificial Sequence
  Description of Artificial Sequence: Synthetic peptide
  misc_feature (1)..(1): May or may not be present
ATITDPNP

SEQ ID NO: 18 - protein, 8 aa, Artificial Sequence
  Description of Artificial Sequence: Synthetic peptide
  misc_feature (1)..(1): May or may not be present
PPHKGLLP

SEQ ID NO: 19 - protein, 9 aa, Artificial Sequence
  Description of Artificial Sequence: Synthetic peptide
  misc_feature (1)..(1): May or may not be present
SVSLPDTHH

SEQ ID NO: 20 - protein, 11 aa, Artificial Sequence
  Description of Artificial Sequence: Synthetic peptide
  misc_feature (1)..(1): May or may not be present
GTHGATPTHSP

SEQ ID NO: 21 - protein, 11 aa, Artificial Sequence
  Description of Artificial Sequence: Synthetic peptide
  misc_feature (1)..(1): May or may not be present
VAPGESSMTSL

SEQ ID NO: 22 - protein, 16 aa, Artificial Sequence
  Description of Artificial Sequence: Synthetic peptide
  misc_feature (1)..(4): May or may not be present
LRGSPISRARPLNPHP

SEQ ID NO: 23 - protein, 15 aa, Artificial Sequence
  Description of Artificial Sequence: Synthetic peptide
  misc_feature (1)..(4): May or may not be present
LRGSISRARPLNPHP

SEQ ID NO: 24 - protein, 15 aa, Artificial Sequence
  Description of Artificial Sequence: Synthetic peptide
  misc_feature (1)..(4): May or may not be present
LRGSPSRARPLNPHP

SEQ ID NO: 25 - protein, 14 aa, Artificial Sequence
  Description of Artificial Sequence: Synthetic peptide
  misc_feature (1)..(4): May or may not be present
LRGSSRARPLNPHP

SEQ ID NO: 26 - protein, 16 aa, Artificial Sequence
  Description of Artificial Sequence: Synthetic peptide
  misc_feature (1)..(4): May or may not be present
LRGSYAPMPPLALASP

SEQ ID NO: 27 - protein, 15 aa, Artificial Sequence
  Description of Artificial Sequence: Synthetic peptide
  misc_feature (1)..(4): May or may not be present
LRGSAPMPPLALASP

SEQ ID NO: 28 - protein, 14 aa, Artificial Sequence
  Description of Artificial Sequence: Synthetic peptide
  misc_feature (1)..(4): May or may not be present
LRGSPMPPLALASP

SEQ ID NO: 29 - protein, 13 aa, Artificial Sequence
  Description of Artificial Sequence: Synthetic peptide
  misc_feature (1)..(4): May or may not be present
LRGSMPPLALASP

SEQ ID NO: 30 - protein, 12 aa, Artificial Sequence
  Description of Artificial Sequence: Synthetic peptide
HLPKPANPFPLD

SEQ ID NO: 31 - protein, 5 aa, Artificial Sequence
  Description of Artificial Sequence: Synthetic peptide
PKPAN

SEQ ID NO: 32 - protein, 6 aa, Artificial Sequence
  Description of Artificial Sequence: Synthetic peptide
RARPLN

SEQ ID NO: 33 - protein, 6 aa, Artificial Sequence
  Description of Artificial Sequence: Synthetic peptide
PMPPLA

SEQ ID NO: 34 - protein, 5 aa, Artificial Sequence
  Description of Artificial Sequence: Synthetic peptide
PPPRP

SEQ ID NO: 35 - protein, 4 aa, Artificial Sequence
  Description of Artificial Sequence: Synthetic peptide
LRGS

SEQ ID NO: 36 - protein, 7 aa, Artificial Sequence
  Description of Artificial Sequence: Synthetic peptide
KSEAAAR

SEQ ID NO: 37 - protein, 12 aa, Artificial Sequence
  Description of Artificial Sequence: Synthetic peptide
ELEEKKSELRHK

SEQ ID NO: 38 - protein, 5 aa, Artificial Sequence
  Description of Artificial Sequence: Synthetic peptide
  MOD_RES (2)..(4): Any amino acid that forms an alpha helix; See specification as filed for detailed description of substitutions and preferred embodiments
EXXXR

SEQ ID NO: 39 - protein, 5 aa, Artificial Sequence
  Description of Artificial Sequence: Synthetic peptide
  MOD_RES (2)..(4): Any amino acid that forms an alpha helix; See specification as filed for detailed description of substitutions and preferred embodiments
EXXXK

SEQ ID NO: 40 - protein, 5 aa, Artificial Sequence
  Description of Artificial Sequence: Synthetic peptide
EAAAR

SEQ ID NO: 41 - protein, 9 aa, Unknown
  Description of Unknown: "LAGLIDADG" family peptide motif sequence
LAGLIDADG

SEQ ID NO: 42 - DNA, 25 bp, Homo sapiens
ctgacctcttctcttcctcccacag

SEQ ID NO: 43 - DNA, 13 bp, Homo sapiens
tttctctccacag

SEQ ID NO: 44 - protein, 16 aa, Artificial Sequence
  Description of Artificial Sequence: Synthetic peptide
LRGSQLVKSELEEKKS

SEQ ID NO: 45 - protein, 29 aa, Artificial Sequence
  Description of Artificial Sequence: Synthetic peptide
HAQRCNGSYAPMPPLALASPELEEKKSEL

SEQ ID NO: 46 - protein, 29 aa, Artificial Sequence
  Description of Artificial Sequence: Synthetic peptide
HTKIHNGSYAPMPPLALASPELEEKKSEL

SEQ ID NO: 47 - protein, 29 aa, Artificial Sequence
  Description of Artificial Sequence: Synthetic peptide
HTKIHGGSYAPMPPLALASPELEEKKSEL

SEQ ID NO: 48 - protein, 28 aa, Artificial Sequence
  Description of Artificial Sequence: Synthetic peptide
HTKIHGSYAPMPPLALASPELEEKKSEL

SEQ ID NO: 49 - protein, 30 aa, Artificial Sequence
  Description of Artificial Sequence: Synthetic polypeptide
HTKIHLRGSYAPMPPLALASPELEEKKSEL

SEQ ID NO: 50 - protein, 9 aa, Artificial Sequence
  Description of Artificial Sequence: Synthetic peptide
HTKIHLRGS

SEQ ID NO: 51 - protein, 19 aa, Artificial Sequence
  Description of Artificial Sequence: Synthetic peptide
HTKIHLRGSQLVKSELEEK

SEQ ID NO: 52 - protein, 31 aa, Artificial Sequence
  Description of Artificial Sequence: Synthetic polypeptide
MAERPFQCRICMRNFSRSDNLGVHIRTHTGE

SEQ ID NO: 53 - protein, 28 aa, Artificial Sequence
  Description of Artificial Sequence: Synthetic peptide
KPFACDICGRKFAQKINLQVHTKIHTGE

SEQ ID NO: 54 - protein, 28 aa, Artificial Sequence
  Description of Artificial Sequence: Synthetic peptide
KPFQCRICMRNFSRSDVLSEHIRTHTGE

SEQ ID NO: 55 - protein, 40 aa, Artificial Sequence
  Description of Artificial Sequence: Synthetic polypeptide
KPFACDICGRKFAQRNHRTTHAQRCGLRGSQLVKSELEEK

SEQ ID NO: 56 - DNA, 31 bp, Artificial Sequence
  Description of Artificial Sequence: Synthetic oligonucleotide
ccttttgcagtttatgataaactgcaaaagg

SEQ ID NO: 57 - DNA, 32 bp, Artificial Sequence
  Description of Artificial Sequence: Synthetic oligonucleotide
ccttttgcagtttatgcataaactgcaaaagg

SEQ ID NO: 58 - DNA, 33 bp, Artificial Sequence
  Description of Artificial Sequence: Synthetic oligonucleotide
ccttttgcagtttatgacataaactgcaaaagg

SEQ ID NO: 59 - DNA, 34 bp, Artificial Sequence
  Description of Artificial Sequence: Synthetic oligonucleotide
ccttttgcagtttatgagcataaactgcaaaagg

SEQ ID NO: 60 - DNA, 41 bp, Artificial Sequence
  Description of Artificial Sequence: Synthetic oligonucleotide
ccttttgcagtttatgagtaccgatcataaactgcaaaagg

SEQ ID NO: 61 - DNA, 42 bp, Artificial Sequence
  Description of Artificial Sequence: Synthetic oligonucleotide
ccttttgcagtttatgagtacgcgatcataaactgcaaaagg

SEQ ID NO: 62 - protein, 8 aa, Artificial Sequence
  Description of Artificial Sequence: Synthetic peptide
TRNPGTVS

SEQ ID NO: 63 - protein, 8 aa, Artificial Sequence
  Description of Artificial Sequence: Synthetic peptide
HVARRKSN

SEQ ID NO: 64 - protein, 8 aa, Artificial Sequence
  Description of Artificial Sequence: Synthetic peptide
PSTIPYNF

SEQ ID NO: 65 - protein, 9 aa, Artificial Sequence
  Description of Artificial Sequence: Synthetic peptide
HPPANSPTP

SEQ ID NO: 66 - protein, 9 aa, Artificial Sequence
  Description of Artificial Sequence: Synthetic peptide
HPLPPIRPV

SEQ ID NO: 67 - protein, 9 aa, Artificial Sequence
  Description of Artificial Sequence: Synthetic peptide
HVSHRSTPI

SEQ ID NO: 68 - protein, 9 aa, Artificial Sequence
  Description of Artificial Sequence: Synthetic peptide
PRPIRHPLP

SEQ ID NO: 69 - protein, 9 aa, Artificial Sequence
  Description of Artificial Sequence: Synthetic peptide
PAARLHPAS

SEQ ID NO: 70 - protein, 9 aa, Artificial Sequence
  Description of Artificial Sequence: Synthetic peptide
PASPALSHT

SEQ ID NO: 71 - protein, 9 aa, Artificial Sequence
  Description of Artificial Sequence: Synthetic peptide
LGKDQNRIP

SEQ ID NO: 72 - protein, 10 aa, Artificial Sequence
  Description of Artificial Sequence: Synthetic peptide
TMPFARLRLT

SEQ ID NO: 73 - protein, 10 aa, Artificial Sequence
  Description of Artificial Sequence: Synthetic peptide
TSTLLVYRAA

SEQ ID NO: 74 - protein, 10 aa, Artificial Sequence
  Description of Artificial Sequence: Synthetic peptide
SYASTSCMPL

SEQ ID NO: 75 - protein, 10 aa, Artificial Sequence
  Description of Artificial Sequence: Synthetic peptide
RTKTLPPPRP

SEQ ID NO: 76 - protein, 11 aa, Artificial Sequence
  Description of Artificial Sequence: Synthetic peptide
IPHNRPRLTVL

SEQ ID NO: 77 - protein, 11 aa, Artificial Sequence
  Description of Artificial Sequence: Synthetic peptide
RARQRLRSAFP

SEQ ID NO: 78 - protein, 11 aa, Artificial Sequence
  Description of Artificial Sequence: Synthetic peptide
GTHGATPTHSP

SEQ ID NO: 79 - protein, 11 aa, Artificial Sequence
  Description of Artificial Sequence: Synthetic peptide
FDSMITAAPFI

SEQ ID NO: 80 - protein, 12 aa, Artificial Sequence
  Description of Artificial Sequence: Synthetic peptide
TRFGIRSYPHED

SEQ ID NO: 81 - protein, 12 aa, Artificial Sequence
  Description of Artificial Sequence: Synthetic peptide
SLSSQPTLVLCT

SEQ ID NO: 82 - protein, 12 aa, Artificial Sequence
  Description of Artificial Sequence: Synthetic peptide
RTLGPSCAADHT

SEQ ID NO: 83 - protein, 12 aa, Artificial Sequence
  Description of Artificial Sequence: Synthetic peptide
DVPNQPDRVHTT

SEQ ID NO: 84 - protein, 12 aa, Artificial Sequence
  Description of Artificial Sequence: Synthetic peptide
GVPPHMSHDCNT

SEQ ID NO: 85 - protein, 13 aa, Artificial Sequence
  Description of Artificial Sequence: Synthetic peptide
NSTYSSTRPISRP

SEQ ID NO: 86 - protein, 13 aa, Artificial Sequence
  Description of Artificial Sequence: Synthetic peptide
RAQQLFAKPTHPI

SEQ ID NO: 87 - protein, 13 aa, Artificial Sequence
  Description of Artificial Sequence: Synthetic peptide
CPGQSRNVFSTPP

SEQ ID NO: 88 - protein, 14 aa, Artificial Sequence
  Description of Artificial Sequence: Synthetic peptide
TRAISRDPVNIRIH

SEQ ID NO: 89 - protein, 14 aa, Artificial Sequence
  Description of Artificial Sequence: Synthetic peptide
SVATHPEGAATPPR

SEQ ID NO: 90 - protein, 15 aa, Artificial Sequence
  Description of Artificial Sequence: Synthetic peptide
LINLHARNSVAYHPV

SEQ ID NO: 91 - protein, 8 aa, Artificial Sequence
  Description of Artificial Sequence: Synthetic peptide
HDMPRHPF

SEQ ID NO: 92 - protein, 8 aa, Artificial Sequence
  Description of Artificial Sequence: Synthetic peptide
QKQPQAHR

SEQ ID NO: 93 - protein, 9 aa, Artificial Sequence
  Description of Artificial Sequence: Synthetic peptide
NLLPPIAGS

SEQ ID NO: 94 - protein, 9 aa, Artificial Sequence
  Description of Artificial Sequence: Synthetic peptide
HPRTRSHYP

SEQ ID NO: 95 - protein, 9 aa, Artificial Sequence
  Description of Artificial Sequence: Synthetic peptide
PRVLINPLV

SEQ ID NO: 96 - protein, 9 aa, Artificial Sequence
  Description of Artificial Sequence: Synthetic peptide
LSPAQSFPH

SEQ ID NO: 97 - protein, 9 aa, Artificial Sequence
  Description of Artificial Sequence: Synthetic peptide
VRQTKNRAE

SEQ ID NO: 98 - protein, 9 aa, Artificial Sequence
  Description of Artificial Sequence: Synthetic peptide
YTTPPPRVP

SEQ ID NO: 99 - protein, 10 aa, Artificial Sequence
  Description of Artificial Sequence: Synthetic peptide
NNSCGDSPRH

SEQ ID NO: 100 - protein, 10 aa, Artificial Sequence
  Description of Artificial Sequence: Synthetic peptide
KLGPLPQIPP

SEQ ID NO: 101 - protein, 10 aa, Artificial Sequence
  Description of Artificial Sequence: Synthetic peptide
TSSLRPHAYH

SEQ ID NO: 102 - protein, 10 aa, Artificial Sequence
  Description of Artificial Sequence: Synthetic peptide
HCPASRPIHP

SEQ ID NO: 103 - protein, 10 aa, Artificial Sequence
  Description of Artificial Sequence: Synthetic peptide
RPFLVAHTPI

SEQ ID NO: 104 - protein, 10 aa, Artificial Sequence
  Description of Artificial Sequence: Synthetic peptide
VPNQFRDDVY

SEQ ID NO: 105 - protein, 10 aa, Artificial Sequence
  Description of Artificial Sequence: Synthetic peptide
SLHTTSRRSI

SEQ ID NO: 106 - protein, 11 aa, Artificial Sequence
  Description of Artificial Sequence: Synthetic peptide
NTYYPSPPLPT

SEQ ID NO: 107 - protein, 11 aa, Artificial Sequence
  Description of Artificial Sequence: Synthetic peptide
SLSATNPPFLN

SEQ ID NO: 108 - protein, 11 aa, Artificial Sequence
  Description of Artificial Sequence: Synthetic peptide
GLQSLIPQQLL

SEQ ID NO: 109 - protein, 11 aa, Artificial Sequence
  Description of Artificial Sequence: Synthetic peptide
VLPKPMCNPPS

SEQ ID NO: 110 - protein, 11 aa, Artificial Sequence
  Description of Artificial Sequence: Synthetic peptide
SPDLTNRSHSL

SEQ ID NO: 111 - protein, 11 aa, Artificial Sequence
  Description of Artificial Sequence: Synthetic peptide
SYLANLPYPHL

SEQ ID NO: 112 - protein, 12 aa, Artificial Sequence
  Description of Artificial Sequence: Synthetic peptide
KHHAPPIMSRPA

SEQ ID NO: 113 - protein, 12 aa, Artificial Sequence
  Description of Artificial Sequence: Synthetic peptide
RPAHHRPAGIPR

SEQ ID NO: 114 - protein, 12 aa, Artificial Sequence
  Description of Artificial Sequence: Synthetic peptide
PTPTLHDAYAPS

SEQ ID NO: 115 - protein, 12 aa, Artificial Sequence
  Description of Artificial Sequence: Synthetic peptide
PTAYPSRPTFTS

SEQ ID NO: 116 - protein, 12 aa, Artificial Sequence
  Description of Artificial Sequence: Synthetic peptide
PPSPPKNLNHRV

SEQ ID NO: 117 - protein, 12 aa, Artificial Sequence
  Description of Artificial Sequence: Synthetic peptide
FRSSHNPVPFTP

SEQ ID NO: 118 - protein, 13 aa, Artificial Sequence
  Description of Artificial Sequence: Synthetic peptide
TSRSSHPVLTIPS

SEQ ID NO: 119 - protein, 13 aa, Artificial Sequence
  Description of Artificial Sequence: Synthetic peptide
PSTGADHTPLPSA

SEQ ID NO: 120 - protein, 14 aa, Artificial Sequence
  Description of Artificial Sequence: Synthetic peptide
NQINPPDDTAVSKY

SEQ ID NO: 121 - protein, 13 aa, Artificial Sequence
  Description of Artificial Sequence: Synthetic peptide
ARPQPLHSRVHLH

SEQ ID NO: 122 - protein, 14 aa, Artificial Sequence
  Description of Artificial Sequence: Synthetic peptide
HRDGPRNLPPTSPP

SEQ ID NO: 123 - protein, 14 aa, Artificial Sequence
  Description of Artificial Sequence: Synthetic peptide
PTRHPRAPSSAAFH

SEQ ID NO: 124 - protein, 14 aa, Artificial Sequence
  Description of Artificial Sequence: Synthetic peptide
PTAQPHKAHPPHWP

SEQ ID NO: 125 - protein, 14 aa, Artificial Sequence
  Description of Artificial Sequence: Synthetic peptide
RNTTPIPPSGGPEP

SEQ ID NO: 126 - protein, 14 aa, Artificial Sequence
  Description of Artificial Sequence: Synthetic peptide
RGIQHKTQRTHPSP

SEQ ID NO: 127 - protein, 14 aa, Artificial Sequence
  Description of Artificial Sequence: Synthetic peptide
LGSVLPSPRWLPGP

SEQ ID NO: 128 - protein, 14 aa, Artificial Sequence
  Description of Artificial Sequence: Synthetic peptide
DPTSTRSSDVKFSP

SEQ ID NO: 129 - protein, 14 aa, Artificial Sequence
  Description of Artificial Sequence: Synthetic peptide
ARNGAPRPRLNILN

SEQ ID NO: 130 - protein, 14 aa, Artificial Sequence
  Description of Artificial Sequence: Synthetic peptide
GSVKHRPMPHRHPA

SEQ ID NO: 131 - protein, 14 aa, Artificial Sequence
  Description of Artificial Sequence: Synthetic peptide
GVRRTSRLDLNAQS

SEQ ID NO: 132 - protein, 15 aa, Artificial Sequence
  Description of Artificial Sequence: Synthetic peptide
NGMAMTQYRPLDHNP

SEQ ID NO: 133 - protein, 15 aa, Artificial Sequence
  Description of Artificial Sequence: Synthetic peptide
NGWNHAFRPAVPSAP

SEQ ID NO: 134 - protein, 15 aa, Artificial Sequence
  Description of Artificial Sequence: Synthetic peptide
TRGLSTPRDVPTVLP

SEQ ID NO: 135 - protein, 15 aa, Artificial Sequence
  Description of Artificial Sequence: Synthetic peptide
TSPDFHPPTTNLSLP

SEQ ID NO: 136 - protein, 15 aa, Artificial Sequence
  Description of Artificial Sequence: Synthetic peptide
PPRPQTGEQITQPSL

SEQ ID NO: 137 - protein, 15 aa, Artificial Sequence
  Description of Artificial Sequence: Synthetic peptide
PGPHTQSQTLRTPSH

SEQ ID NO: 138 - protein, 15 aa, Artificial Sequence
  Description of Artificial Sequence: Synthetic peptide
ARAGTTPPINTLPTR

SEQ ID NO: 139 - protein, 15 aa, Artificial Sequence
  Description of Artificial Sequence: Synthetic peptide
ALYTQGPVRPARTPP

SEQ ID NO: 140 - protein, 15 aa, Artificial Sequence
  Description of Artificial Sequence: Synthetic peptide
GRGLGLTLHRVPNHP

SEQ ID NO: 141 - protein, 15 aa, Artificial Sequence
  Description of Artificial Sequence: Synthetic peptide
GLLYSIPNLARVSHS

SEQ ID NO: 142 - protein, 15 aa, Artificial Sequence
  Description of Artificial Sequence: Synthetic peptide
GFPQPHRRRAALVCP

SEQ ID NO: 143 - protein, 15 aa, Artificial Sequence
  Description of Artificial Sequence: Synthetic peptide
SGSNPTPSRVLTPIT

SEQ ID NO: 144 - protein, 16 aa, Artificial Sequence
  Description of Artificial Sequence: Synthetic peptide
NGHTGHRDKPAALVTR

SEQ ID NO: 145 - protein, 16 aa, Artificial Sequence
  Description of Artificial Sequence: Synthetic peptide
TGIFRILDVSPANGSP

SEQ ID NO: 146 - protein, 16 aa, Artificial Sequence
  Description of Artificial Sequence: Synthetic peptide
PLNAHAPKSRRTLEPP

SEQ ID NO: 147 - protein, 16 aa, Artificial Sequence
  Description of Artificial Sequence: Synthetic peptide
LRPNSLSALRSSSPLI

SEQ ID NO: 148 - protein, 16 aa, Artificial Sequence
  Description of Artificial Sequence: Synthetic peptide
DPNSPISRARPLNPHP

SEQ ID NO: 149 - protein, 12 aa, Artificial Sequence
  Description of Artificial Sequence: Synthetic peptide
QGQAVYDTPPTP

SEQ ID NO: 150 - protein, 14 aa, Artificial Sequence
  Description of Artificial Sequence: Synthetic peptide
NGICPPPRPRTSPP

SEQ ID NO: 151 - protein, 14 aa, Artificial Sequence
  Description of Artificial Sequence: Synthetic peptide
KGVHKATPPASPSY

SEQ ID NO: 152 - protein, 14 aa, Artificial Sequence
  Description of Artificial Sequence: Synthetic peptide
TGTRSPVSTPISHP

SEQ ID NO: 153 - protein, 14 aa, Artificial Sequence
  Description of Artificial Sequence: Synthetic peptide
TGSVHPSRPPLHNS

SEQ ID NO: 154 - protein, 14 aa, Artificial Sequence
  Description of Artificial Sequence: Synthetic peptide
PIISPPLPPSAPLP

SEQ ID NO: 155 - protein, 14 aa, Artificial Sequence
  Description of Artificial Sequence: Synthetic peptide
PGVAPLRPKNRVHP

SEQ ID NO: 156 - protein, 14 aa, Artificial Sequence
  Description of Artificial Sequence: Synthetic peptide
PVTTYTRMAHPTTP

SEQ ID NO: 157 - protein, 14 aa, Artificial Sequence
  Description of Artificial Sequence: Synthetic peptide
LGLNAPVKTPPPLP

SEQ ID NO: 158 - protein, 14 aa, Artificial Sequence
  Description of Artificial Sequence: Synthetic peptide
LGLNAPVTTPPPLP

SEQ ID NO: 159 - protein, 15 aa, Artificial Sequence
  Description of Artificial Sequence: Synthetic peptide
TASAPAMRPVVVQNA

SEQ ID NO: 160 - protein, 15 aa, Artificial Sequence
  Description of Artificial Sequence: Synthetic peptide
TGKNSTSFTTRGTIP

SEQ ID NO: 161 - protein, 15 aa, Artificial Sequence
  Description of Artificial Sequence: Synthetic peptide
TGTVHTSPICPQTYP

SEQ ID NO: 162 - protein, 15 aa, Artificial Sequence
  Description of Artificial Sequence: Synthetic peptide
QGVLRRSFHRPPIVL

SEQ ID NO: 163 - protein, 15 aa, Artificial Sequence
  Description of Artificial Sequence: Synthetic peptide
PHITTRHSQPKTHPV

SEQ ID NO: 164 - protein, 15 aa, Artificial Sequence
  Description of Artificial Sequence: Synthetic peptide
PQFRAPAKPPLHNTR

SEQ ID NO: 165 - protein, 15 aa, Artificial Sequence
  Description of Artificial Sequence: Synthetic peptide
AGERHRVRPTAPPTL

SEQ ID NO: 166 - protein, 15 aa, Artificial Sequence
  Description of Artificial Sequence: Synthetic peptide
SAPVASRLLPPKSLP

SEQ ID NO: 167 - protein, 15 aa, Artificial Sequence
  Description of Artificial Sequence: Synthetic peptide
SSIPPRRTQVRTPTP

SEQ ID NO: 168 - protein, 16 aa, Artificial Sequence
  Description of Artificial Sequence: Synthetic peptide
NGSQTPKRFQPTHPSA

SEQ ID NO: 169 - protein, 16 aa, Artificial Sequence
  Description of Artificial Sequence: Synthetic peptide
PTRPSPSGLNTPVPNP

SEQ ID NO: 170 - protein, 17 aa, Artificial Sequence
  Description of Artificial Sequence: Synthetic peptide
PKLDTPTAHTPVSRTSP

SEQ ID NO: 171 - protein, 17 aa, Artificial Sequence
  Description of Artificial Sequence: Synthetic peptide
PNLRPSPHVNSSPPHSS

SEQ ID NO: 172 - protein, 8 aa, Artificial Sequence
  Description of Artificial Sequence: Synthetic peptide
TNKRTNLS

SEQ ID NO: 173 - protein, 8 aa, Artificial Sequence
  Description of Artificial Sequence: Synthetic peptide
TPAPIPTS

SEQ ID NO: 174 - protein, 8 aa, Artificial Sequence
  Description of Artificial Sequence: Synthetic peptide
TPNAKLPH

SEQ ID NO: 175 - protein, 8 aa, Artificial Sequence
  Description of Artificial Sequence: Synthetic peptide
HPIHPGIY

SEQ ID NO: 176 - protein, 8 aa, Artificial Sequence
  Description of Artificial Sequence: Synthetic peptide
HPRKPVPF

SEQ ID NO: 177 - protein, 8 aa, Artificial Sequence
  Description of Artificial Sequence: Synthetic peptide
HGPRHTPV

SEQ ID NO: 178 - protein, 8 aa, Artificial Sequence
  Description of Artificial Sequence: Synthetic peptide
GVAAASPP

SEQ ID NO: 179 - protein, 9 aa, Artificial Sequence
  Description of Artificial Sequence: Synthetic peptide
NIRNYNAAA

SEQ ID NO: 180 - protein, 9 aa, Artificial Sequence
  Description of Artificial Sequence: Synthetic peptide
PPPHSPPPF

SEQ ID NO: 181 - protein, 9 aa, Artificial Sequence
  Description of Artificial Sequence: Synthetic peptide
PFPYSSPHH

SEQ ID NO: 182 - protein, 9 aa, Artificial Sequence
  Description of Artificial Sequence: Synthetic peptide
LPARPGIPH

SEQ ID NO: 183 - protein, 9 aa, Artificial Sequence
  Description of Artificial Sequence: Synthetic peptide
LCCHSRPAN

SEQ ID NO: 184 - protein, 9 aa, Artificial Sequence
  Description of Artificial Sequence: Synthetic peptide
LPNMTLKPY

SEQ ID NO: 185 - protein, 10 aa, Artificial Sequence
  Description of Artificial Sequence: Synthetic peptide
TDSRHRRSII

SEQ ID NO: 186 - protein, 10 aa, Artificial Sequence
  Description of Artificial Sequence: Synthetic peptide
RPSHFRPVPP

SEQ ID NO: 187 - protein, 10 aa, Artificial Sequence
  Description of Artificial Sequence: Synthetic peptide
FTPGHHHPHT

SEQ ID NO: 188 - protein, 10 aa, Artificial Sequence
  Description of Artificial Sequence: Synthetic peptide
FSTPNTPRIN

SEQ ID NO: 189 - protein, 11 aa, Artificial Sequence
  Description of Artificial Sequence: Synthetic peptide
SVTGSHTRDTI

SEQ ID NO: 190 - protein, 11 aa, Artificial Sequence
  Description of Artificial Sequence: Synthetic peptide
SLFPLRPHLPP

SEQ ID NO: 191 - protein, 12 aa, Artificial Sequence
  Description of Artificial Sequence: Synthetic peptide
KSPEAPNPIAFP

SEQ ID NO: 192 - protein, 12 aa, Artificial Sequence
  Description of Artificial Sequence: Synthetic peptide
TPLLRTHVGFPR

SEQ ID NO: 193 - protein, 12 aa, Artificial Sequence
  Description of Artificial Sequence: Synthetic peptide
SSLVMADPHYQF

SEQ ID NO: 194 - protein, 15 aa, Artificial Sequence
  Description of Artificial Sequence: Synthetic peptide
PLANSTSAHPARMPE

SEQ ID NO: 195 - protein, 15 aa, Artificial Sequence
  Description of Artificial Sequence: Synthetic peptide
APACHTTPNAPRYPL

SEQ ID NO: 196 - protein, 15 aa, Artificial Sequence
  Description of Artificial Sequence: Synthetic peptide
GNTLTIRSEQDLVVI

SEQ ID NO: 197 - protein, 15 aa, Artificial Sequence
  Description of Artificial Sequence: Synthetic peptide
YHTPLNYPLLPDHYY

SEQ ID NO: 198 - protein, 16 aa, Artificial Sequence
  Description of Artificial Sequence: Synthetic peptide
HSPRRSDPPAPHSDEA

SEQ ID NO: 199 - protein, 8 aa, Artificial Sequence
  Description of Artificial Sequence: Synthetic peptide
HPPQHFGH

SEQ ID NO: 200 - protein, 9 aa, Artificial Sequence
  Description of Artificial Sequence: Synthetic peptide
HSKTTNLTP

SEQ ID NO: 201 - protein, 9 aa, Artificial Sequence
  Description of Artificial Sequence: Synthetic peptide
GATPTKLLP

SEQ ID NO: 202 - protein, 10 aa, Artificial Sequence
  Description of Artificial Sequence: Synthetic peptide
NRRSSPRPRT

SEQ ID NO: 203 - protein, 10 aa, Artificial Sequence
  Description of Artificial Sequence: Synthetic peptide
HSNFQDIKEI

SEQ ID NO: 204 - protein, 10 aa, Artificial Sequence
  Description of Artificial Sequence: Synthetic peptide
PLFPQPELPC

SEQ ID NO: 205 - protein, 11 aa, Artificial Sequence
  Description of Artificial Sequence: Synthetic peptide
SRPKYPTPHLD

SEQ ID NO: 206 - protein, 11 aa, Artificial Sequence
  Description of Artificial Sequence: Synthetic peptide
GTNKYPFVAHL

SEQ ID NO: 207 - protein, 11 aa, Artificial Sequence
  Description of Artificial Sequence: Synthetic peptide
GSSHDTRRPHV

SEQ ID NO: 208 - protein, 11 aa, Artificial Sequence
  Description of Artificial Sequence: Synthetic peptide
GARLPAGHNHT

SEQ ID NO: 209 - protein, 11 aa, Artificial Sequence
  Description of Artificial Sequence: Synthetic peptide
SLLPLAPKYHF

SEQ ID NO: 210 - protein, 12 aa, Artificial Sequence
  Description of Artificial Sequence: Synthetic peptide
SIPDLPVFSTIP

SEQ ID NO: 211 - protein, 12 aa, Artificial Sequence
  Description of Artificial Sequence: Synthetic peptide
ALPPTPSFPPPW

SEQ ID NO: 212 - protein, 13 aa, Artificial Sequence
  Description of Artificial Sequence: Synthetic peptide
PSLDTPAIIPTVH

SEQ ID NO: 213 - protein, 13 aa, Artificial Sequence
  Description of Artificial Sequence: Synthetic peptide
PHRGASSTQCLSH

SEQ ID NO: 214 - protein, 13 aa, Artificial Sequence
  Description of Artificial Sequence: Synthetic peptide
PSRSPASTLSPRH

SEQ ID NO: 215 - protein, 14 aa, Artificial Sequence
  Description of Artificial Sequence: Synthetic peptide
PVAHPRPDLHPTTT

SEQ ID NO: 216 - protein, 14 aa, Artificial Sequence
  Description of Artificial Sequence: Synthetic peptide
AARHQNDLTSPAYS

SEQ ID NO: 217 - protein, 14 aa, Artificial Sequence
  Description of Artificial Sequence: Synthetic peptide
GTNPPNTNPRHSHY

SEQ ID NO: 218 - protein, 14 aa, Artificial Sequence
  Description of Artificial Sequence: Synthetic peptide
GPAKSPPNPSSTRV

SEQ ID NO: 219 - protein, 15 aa, Artificial Sequence
  Description of Artificial Sequence: Synthetic peptide
KNSILDPRSATRAHL

SEQ ID NO: 220 - protein, 15 aa, Artificial Sequence
  Description of Artificial Sequence: Synthetic peptide
PKPPPLFSSPRINNP

SEQ ID NO: 221 - protein, 15 aa, Artificial Sequence
  Description of Artificial Sequence: Synthetic peptide
RVGTHPASSVRSDWP

SEQ ID NO: 222 - protein, 16 aa, Artificial Sequence
  Description of Artificial Sequence: Synthetic peptide
VNSDPLASAPRREPRL

SEQ ID NO: 223 - protein, 16 aa, Artificial Sequence
  Description of Artificial Sequence: Synthetic peptide
SSNRPNPHATKWMPTH

SEQ ID NO: 224 - protein, 16 aa, Artificial Sequence
  Description of Artificial Sequence: Synthetic peptide
SQPKATTSARRPNTTT

SEQ ID NO: 225 - protein, 17 aa, Artificial Sequence
  Description of Artificial Sequence: Synthetic peptide
TRSTSHKARDDTRPIPC

SEQ ID NO: 226 - protein, 17 aa, Artificial Sequence
  Description of Artificial Sequence: Synthetic peptide
RHAANPPSRHCRTAPHP

SEQ ID NO: 227 - DNA, 29 bp, Artificial Sequence
  Description of Artificial Sequence: Synthetic oligonucleotide
gtcatcctcatccgtttaaactgcaaaag

SEQ ID NO: 228 - DNA, 30 bp, Artificial Sequence
  Description of Artificial Sequence: Synthetic oligonucleotide
gtcatcctcatcctgtttaaactgcaaaag

SEQ ID NO: 229 - DNA, 31 bp, Artificial Sequence
  Description of Artificial Sequence: Synthetic oligonucleotide
gtcatcctcatcctggtttaaactgcaaaag

SEQ ID NO: 230 - DNA, 32 bp, Artificial Sequence
  Description of Artificial Sequence: Synthetic oligonucleotide
gtcatcctcatcctgagtttaaactgcaaaag

SEQ ID NO: 231 - DNA, 39 bp, Artificial Sequence
  Description of Artificial Sequence: Synthetic oligonucleotide
gtcatcctcatcctgatactgctgtttaaactgcaaaag

SEQ ID NO: 232 - DNA, 40 bp, Artificial Sequence
  Description of Artificial Sequence: Synthetic oligonucleotide
gtcatcctcatcctgatactagctgtttaaactgcaaaag

SEQ ID NO: 233 - protein, 17 aa, Artificial Sequence
  Description of Artificial Sequence: Synthetic peptide
GLRGSQLVKSKSEAAAR

SEQ ID NO: 234 - protein, 17 aa, Artificial Sequence
  Description of Artificial Sequence: Synthetic peptide
TGLMPPSHPRQPIHINF

SEQ ID NO: 235 - protein, 15 aa, Artificial Sequence
  Description of Artificial Sequence: Synthetic peptide
TGSGTPTRPHPPLPP

SEQ ID NO: 236 - protein, 15 aa, Artificial Sequence
  Description of Artificial Sequence: Synthetic peptide
GRPRRPTDTPLGSPP

SEQ ID NO: 237 - protein, 10 aa, Artificial Sequence
  Description of Artificial Sequence: Synthetic peptide
HTTPNPHANT

SEQ ID NO: 238 - protein, 9 aa, Artificial Sequence
  Description of Artificial Sequence: Synthetic peptide
ILTPVTHVV

SEQ ID NO: 239 - protein, 9 aa, Artificial Sequence
  Description of Artificial Sequence: Synthetic peptide
HRILSPSRG

SEQ ID NO: 240 - protein, 11 aa, Artificial Sequence
  Description of Artificial Sequence: Synthetic peptide
GTPRASSDSSF

SEQ ID NO: 241 - DNA, 75 bp, Artificial Sequence
  Description of Artificial Sequence: Synthetic oligonucleotide
  CDS (1)..(15)
  CDS (55)..(75)
atccacggggtaccgagaccggcattaagcttgatatctcaggccacggtctccgagctggaggagaagaagtcc

SEQ ID NO: 242 - protein, 12 aa, Artificial Sequence
  Description of Artificial Sequence: Synthetic peptide
IHGVPELEEKKS

SEQ ID NO: 243 - DNA, 48 bp, Artificial Sequence
  Description of Artificial Sequence: Synthetic oligonucleotide
  CDS (1)..(48)
agatgcaacggtatctgcccacctccaaggcccaggacctccccacca

SEQ ID NO: 244 - protein, 16 aa, Artificial Sequence
  Description of Artificial Sequence: Synthetic peptide
RCNGICPPPRPRTSPP

SEQ ID NO: 245 - DNA, 51 bp, Artificial Sequence
  Description of Artificial Sequence: Synthetic oligonucleotide
  CDS (1)..(51)
agatgcaacggttcctacgctccaatgccacccctggctctggcttcccca

SEQ ID NO: 246 - protein, 17 aa, Artificial Sequence
  Description of Artificial Sequence: Synthetic peptide
RCNGSYAPMPPLALASP

SEQ ID NO: 247 - DNA, 51 bp, Artificial Sequence
  Description of Artificial Sequence: Synthetic oligonucleotide
  CDS (1)..(51)
agatgcccaggtatctacaccgctccaacctccaggccaaccgtgcctcca

SEQ ID NO: 248 - protein, 17 aa, Artificial Sequence
  Description of Artificial Sequence: Synthetic peptide
RCPGIYTAPTSRPTVPP

SEQ ID NO: 249 - DNA, 57 bp, Artificial Sequence
  Description of Artificial Sequence: Synthetic oligonucleotide
  CDS (1)..(57)
agatgcaccggcctgatgccaccctcccacccaaggcagccaatccacatcaacttc

SEQ ID NO: 250 - protein, 19 aa, Artificial Sequence
  Description of Artificial Sequence: Synthetic peptide
RCTGLMPPSHPRQPIHINF

SEQ ID NO: 251 - DNA, 45 bp, Artificial Sequence
  Description of Artificial Sequence: Synthetic oligonucleotide
  CDS (1)..(45)
cataccaagatacacctgcgccaaaaagatgcggcccggggatcc

SEQ ID NO: 252 - protein, 15 aa, Artificial Sequence
  Description of Artificial Sequence: Synthetic peptide
HTKIHLRQKDAARGS

SEQ ID NO: 253 - DNA, 39 bp, Artificial Sequence
  Description of Artificial Sequence: Synthetic oligonucleotide
  CDS (1)..(15)
cataccaagatatgccgagacgaaaaagatgcggcccgg

SEQ ID NO: 254 - protein, 5 aa, Artificial Sequence
  Description of Artificial Sequence: Synthetic peptide
HTKIC

SEQ ID NO: 255 - DNA, 39 bp, Artificial Sequence
  Description of Artificial Sequence: Synthetic oligonucleotide
  CDS (1)..(15)
catgcccagagatgccgagaccaaaaagatgcggcccgg

SEQ ID NO: 256 - protein, 5 aa, Artificial Sequence
  Description of Artificial Sequence: Synthetic peptide
HAQRC

SEQ ID NO: 257 - DNA, 15 bp, Artificial Sequence
  Description of Artificial Sequence: Synthetic oligonucleotide
  CDS (1)..(15)
catgcccagagatgc

SEQ ID NO: 258 - protein, 22 aa, Artificial Sequence
  Description of Artificial Sequence: Synthetic peptide
HAQRCHLPKPANPFPLDELEEK

SEQ ID NO: 259 - protein, 26 aa, Artificial Sequence
  Description of Artificial Sequence: Synthetic peptide
HAQRCDPNSPISRARPLNPHPELEEK

SEQ ID NO: 260 - protein, 24 aa, Artificial Sequence
  Description of Artificial Sequence: Synthetic peptide
HAQRCNGICPPPRPRTSPPELEEK

SEQ ID NO: 261 - protein, 25 aa, Artificial Sequence
  Description of Artificial Sequence: Synthetic peptide
HAQRCNGSYAPMPPLALASPELEEK

SEQ ID NO: 262 - protein, 22 aa, Artificial Sequence
  Description of Artificial Sequence: Synthetic peptide
HTKIHHLPKPANPFPLDELEEK

SEQ ID NO: 263 - protein, 26 aa, Artificial Sequence
  Description of Artificial Sequence: Synthetic peptide
HTKIHDPNSPISRARPLNPHPELEEK

SEQ ID NO: 264 - protein, 24 aa, Artificial Sequence
  Description of Artificial Sequence: Synthetic peptide
HTKIHNGICPPPRPRTSPPELEEK

SEQ ID NO: 265 - protein, 25 aa, Artificial Sequence
  Description of Artificial Sequence: Synthetic peptide
HTKIHNGSYAPMPPLALASPELEEK

SEQ ID NO: 266 - protein, 21 aa, Artificial Sequence
  Description of Artificial Sequence: Synthetic peptide
HTKIHLPKPANPFPLDELEEK

SEQ ID NO: 267 - protein, 25 aa, Artificial Sequence
  Description of Artificial Sequence: Synthetic peptide
HTKIHPNSPISRARPLNPHPELEEK

SEQ ID NO: 268 - protein, 23 aa, Artificial Sequence
  Description of Artificial Sequence: Synthetic peptide
HTKIHGICPPPRPRTSPPELEEK

SEQ ID NO: 269 - protein, 24 aa, Artificial Sequence
  Description of Artificial Sequence: Synthetic peptide
HTKIHGSYAPMPPLALASPELEEK

SEQ ID NO: 270 - protein, 26 aa, Artificial Sequence
  Description of Artificial Sequence: Synthetic peptide
HTKIHLRGSQLVKSKSEAAARELEEK

SEQ ID NO: 271 - protein, 26 aa, Artificial Sequence
  Description of Artificial Sequence: Synthetic peptide
HTKIHLRGSQLVKSKSEAAARELEEK

SEQ ID NO: 272 - protein, 26 aa, Artificial Sequence
  Description of Artificial Sequence: Synthetic peptide
HTKIHLRGSPISRARPLNPHPELEEK

SEQ ID NO: 273 - protein, 25 aa, Artificial Sequence
  Description of Artificial Sequence: Synthetic peptide
HTKIHLRGSISRARPLNPHPELEEK

SEQ ID NO: 274 - protein, 25 aa, Artificial Sequence
  Description of Artificial Sequence: Synthetic peptide
HTKIHLRGSPSRARPLNPHPELEEK

SEQ ID NO: 275 - protein, 24 aa, Artificial Sequence
  Description of Artificial Sequence: Synthetic peptide
HTKIHLRGSSRARPLNPHPELEEK

SEQ ID NO: 276 - protein, 26 aa, Artificial Sequence
  Description of Artificial Sequence: Synthetic peptide
HTKIHLRGSYAPMPPLALASPELEEK

SEQ ID NO: 277 - protein, 25 aa, Artificial Sequence
  Description of Artificial Sequence: Synthetic peptide
HTKIHLRGSAPMPPLALASPELEEK

SEQ ID NO: 278 - protein, 24 aa, Artificial Sequence
  Description of Artificial Sequence: Synthetic peptide
HTKIHLRGSPMPPLALASPELEEK

SEQ ID NO: 279 - protein, 23 aa, Artificial Sequence
  Description of Artificial Sequence: Synthetic peptide
HTKIHLRGSMPPLALASPELEEK

SEQ ID NO: 280 - protein, 16 aa, Artificial Sequence
  Description of Artificial Sequence: Synthetic peptide
HTKIHLRGSKSELEEK

SEQ ID NO: 281 - protein, 17 aa, Artificial Sequence
  Description of Artificial Sequence: Synthetic peptide
HTKIHLRGSGKSELEEK

SEQ ID NO: 282 - protein, 17 aa, Artificial Sequence
  Description of Artificial Sequence: Synthetic peptide
HTKIHLRGSVKSELEEK

SEQ ID NO: 283 - protein, 17 aa, Artificial Sequence
  Description of Artificial Sequence: Synthetic peptide
HTKIHLRGSEKSELEEK

SEQ ID NO: 284 - protein, 18 aa, Artificial Sequence
  Description of Artificial Sequence: Synthetic peptide
HTKIHLRGSGVKSELEEK

SEQ ID NO: 285 - protein, 18 aa, Artificial Sequence
  Description of Artificial Sequence: Synthetic peptide
HTKIHLRGSSVKSELEEK

SEQ ID NO: 286 - protein, 18 aa, Artificial Sequence
  Description of Artificial Sequence: Synthetic peptide
HTKIHLRGSLVKSELEEK

SEQ ID NO: 287 - protein, 18 aa, Artificial Sequence
  Description of Artificial Sequence: Synthetic peptide
HTKIHLRGSEVKSELEEK

SEQ ID NO: 288 - protein, 19 aa, Artificial Sequence
  Description of Artificial Sequence: Synthetic peptide
HTKIHLRGSGLVKSELEEK

SEQ ID NO: 289 - protein, 19 aa, Artificial Sequence
  Description of Artificial Sequence: Synthetic peptide
HTKIHLRGSSLVKSELEEK

SEQ ID NO: 290 - protein, 19 aa, Artificial Sequence
  Description of Artificial Sequence: Synthetic peptide
HTKIHLRGSRLVKSELEEK

SEQ ID NO: 291 - protein, 19 aa, Artificial Sequence
  Description of Artificial Sequence: Synthetic peptide
HTKIHLRGSWLVKSELEEK

SEQ ID NO: 292 - protein, 19 aa, Artificial Sequence
  Description of Artificial Sequence: Synthetic peptide
HTKIHLRGSQGVKSELEEK

SEQ ID NO: 293 - protein, 19 aa, Artificial Sequence
  Description of Artificial Sequence: Synthetic peptide
HTKIHLRGSQSVKSELEEK

SEQ ID NO: 294 - protein, 19 aa, Artificial Sequence
  Description of Artificial Sequence: Synthetic peptide
HTKIHLRGSQLSKSELEEK

SEQ ID NO: 295 - protein, 20 aa, Artificial Sequence
  Description of Artificial Sequence: Synthetic peptide
HTKIHLRGSGQLVKSELEEK

SEQ ID NO: 296 - protein, 20 aa, Artificial Sequence
  Description of Artificial Sequence: Synthetic peptide
HTKIHLRGSSQLVKSELEEK

SEQ ID NO: 297 - protein, 20 aa, Artificial Sequence
  Description of Artificial Sequence: Synthetic peptide
HTKIHLRGSKQLVKSELEEK

SEQ ID NO: 298 - protein, 20 aa, Artificial Sequence
  Description of Artificial Sequence: Synthetic peptide
HTKIHLRGSRQLVKSELEEK

SEQ ID NO: 299 - protein, 21 aa, Artificial Sequence
  Description of Artificial Sequence: Synthetic peptide
HTKIHLRGSGSQLVKSELEEK

SEQ ID NO: 300 - protein, 21 aa, Artificial Sequence
  Description of Artificial Sequence: Synthetic peptide
HTKIHLRGSGKQLVKSELEEK

SEQ ID NO: 301 - protein, 21 aa, Artificial Sequence
  Description of Artificial Sequence: Synthetic peptide
HTKIHLRGSTKQLVKSELEEK

SEQ ID NO: 302 - protein, 22 aa, Artificial Sequence
  Description of Artificial Sequence: Synthetic peptide
HTKIHLRGSGTKQLVKSELEEK

SEQ ID NO: 303 - protein, 22 aa, Artificial Sequence
  Description of Artificial Sequence: Synthetic peptide
HTKIHLRGSVTKQLVKSELEEK

SEQ ID NO: 304 - protein, 4 aa, Artificial Sequence
  Description of Artificial Sequence: Synthetic peptide
GSKS

SEQ ID NO: 305 - protein, 5 aa, Artificial Sequence
  Description of Artificial Sequence: Synthetic peptide
GSVKS

SEQ ID NO: 306 - protein, 6 aa, Artificial Sequence
  Description of Artificial Sequence: Synthetic peptide
GSEVKS

SEQ ID NO: 307 - protein, 7 aa, Artificial Sequence
  Description of Artificial Sequence: Synthetic peptide
GSQSVKS

SEQ ID NO: 308 - protein, 8 aa, Artificial Sequence
  Description of Artificial Sequence: Synthetic peptide
GSKQLVKS

SEQ ID NO: 309 - protein, 9 aa, Artificial Sequence
  Description of Artificial Sequence: Synthetic peptide
GSGKQLVKS

SEQ ID NO: 310 - protein, 10 aa, Artificial Sequence
  Description of Artificial Sequence: Synthetic peptide
GSVTKQLVKS

SEQ ID NO: 311 - protein, 7 aa, Artificial Sequence
  Description of Artificial Sequence: Synthetic peptide
GSQLVKS

SEQ ID NO: 312 - protein, 9 aa, Artificial Sequence
  Description of Artificial Sequence: Synthetic peptide
GSTKQLVKS